European Patent Application EP 4 296 283 A1, published December 27, 2023. Title: Single domain antibodies against PD-L1 and use thereof. Applicant: SNU R&DB Foundation Shaperon. The sequence listing filed with the application follows.

SEQUENCE LISTING (11 sequences)

SEQ ID NO: 1 - protein, 120 aa, Artificial Sequence
  PDL1 Nb#01
QVQLVESGGGLVQPGGSLRLSCAASGFTFSSFAMSWVRQAPGKGLEWVSDINTGGDSTDYADSVKGRFTISRDNAKNTLYLQMNSLKPEDTAVYYCAKGPKEMVHVYSQRGQGTQVTVSS

SEQ ID NO: 2 - protein, 8 aa, Artificial Sequence
  PDL1 Nb#01_CDR1
GFTFSSFA

SEQ ID NO: 3 - protein, 8 aa, Artificial Sequence
  PDL1 Nb#01_CDR2
INTGGDST

SEQ ID NO: 4 - protein, 13 aa, Artificial Sequence
  PDL1 Nb#01_CDR3
AKGPKEMVHVYSQ

SEQ ID NO: 5 - protein, 357 aa, Artificial Sequence
  PDL1 Nb#01-IgG1
QVQLVESGGGLVQPGGSLRLSCAASGFTFSSFAMSWVRQAPGKGLEWVSDINTGGDSTDYADSVKGRFTISRDNAKNTLYLQMNSLKPEDTAVYYCAKGPKEMVHVYSQRGQGTQVTVSSGPGGPEPKSSDKTHTCPPCPAPELLGGPSVFLFPPKPKDTLMISRTPEVTCVVVDVSHEDPEVKFNWYVDGVEVHNAKTKPREEQYNSTYRVVSVLTVLHQDWLNGKEYKCKVSNKALPAPIEKTISKAKGQPREPQVYTLPPSRDELTKNQVSLTCLVKGFYPSDIAVEWESNGQPENNYKTTPPVLDSDGSFFLYSKLTVDKSRWQQGNVFSCSVMHEALHNHYTQKSLSLSPGK

SEQ ID NO: 6 - protein, 25 aa, Artificial Sequence
  PDL1 Nb#01_FR1
QVQLVESGGGLVQPGGSLRLSCAAS

SEQ ID NO: 7 - protein, 17 aa, Artificial Sequence
  PDL1 Nb#01_FR2
MSWVRQAPGKGLEWVSD

SEQ ID NO: 8 - protein, 38 aa, Artificial Sequence
  PDL1 Nb#01_FR3
DYADSVKGRFTISRDNAKNTLYLQMNSLKPEDTAVYYC

SEQ ID NO: 9 - protein, 11 aa, Artificial Sequence
  PDL1 Nb#01_FR4
RGQGTQVTVSS

SEQ ID NO: 10 - protein, 246 aa, Artificial Sequence
  PP Nb
QVQLVESGGGLVQPGGSLRLSCAASGFTFSSFAMSWVRQAPGKGLEWVSDINTGGDSTDYADSVKGRFTISRDNAKNTLYLQMNSLKPEDTAVYYCAKGPKEMVHVYSQRGQGTQVTVSSGGSGGSQVQLVESGGGLVQPGGSLRLSCAASGFTFSSFAMSWVRQAPGKGLEWVSDINTGGDSTDYADSVKGRFTISRDNAKNTLYLQMNSLKPEDTAVYYCAKGPKEMVHVYSQRGQGTQVTVSS

SEQ ID NO: 11 - protein, 480 aa, Artificial Sequence
  PP Nb-IgG4
QVQLVESGGGLVQPGGSLRLSCAASGFTFSSFAMSWVRQAPGKGLEWVSDINTGGDSTDYADSVKGRFTISRDNAKNTLYLQMNSLKPEDTAVYYCAKGPKEMVHVYSQRGQGTQVTVSSGGSGGSQVQLVESGGGLVQPGGSLRLSCAASGFTFSSFAMSWVRQAPGKGLEWVSDINTGGDSTDYADSVKGRFTISRDNAKNTLYLQMNSLKPEDTAVYYCAKGPKEMVHVYSQRGQGTQVTVSSGPGGPESKYGPPCPPCPAPEFLGGPSVFLFPPKPKDTLMISRTPEVTCVVVDVSQEDPEVQFNWYVDGVEVHNAKTKPREEQFNSTYRVVSVLTVLHQDWLNGKEYKCKVSNKGLPSSIEKTISKAKGQPREPQVYTLPPSQEEMTKNQVSLTCLVKGFYPSDIAVEWESNGQPENNYKTTPPVLDSDGSFFLYSRLTVDKSRWQEGNVFSCSVMHEALHNHYTQKSLSLSPGK